European Patent Specification EP 2 801 580 B1, published September 13, 2023. Title: Nucleoside Phosphoramidate Prodrugs. Applicant: Gilead Pharmasset LLC. Application EP14151876.1. The sequence listing filed with the application follows.

SEQUENCE LISTING (3 sequences)

SEQ ID NO: 1 - DNA, 23 bp, Artificial Sequence
  Primer
agccatggcgttagtatgagtgt

SEQ ID NO: 2 - DNA, 18 bp, Artificial Sequence
  Primer
ttccgcagaccactatgg

SEQ ID NO: 3 - DNA, 20 bp, Artificial Sequence
  Primer
cctccaggaccccccctccc